European Patent Application EP 4 382 540 A1, published June 12, 2024. Title: USE OF ANTI-PD-L1/CD47 BISPECIFIC ANTIBODY IN TREATMENT OF DISEASES. Applicant: Bio-Thera Solutions, Ltd. The sequence listing filed with the application follows.

SEQUENCE LISTING (22 sequences)

SEQ ID NO: 1 - protein, 10 aa, synthetic construct
GFTFSDSWIH

SEQ ID NO: 2 - protein, 18 aa, synthetic construct
GWISPYGGSTYYADSYRS

SEQ ID NO: 3 - protein, 9 aa, synthetic construct
RHWPGGFDY

SEQ ID NO: 4 - protein, 11 aa, synthetic construct
LASQTIGTWLA

SEQ ID NO: 5 - protein, 7 aa, synthetic construct
AASTLQS

SEQ ID NO: 6 - protein, 9 aa, synthetic construct
QQYYSTPRT

SEQ ID NO: 7 - protein, 6 aa, synthetic construct
DNYYWS

SEQ ID NO: 8 - protein, 16 aa, synthetic construct
YIYYSGNTNYNPSLKS

SEQ ID NO: 9 - protein, 8 aa, synthetic construct
GGRFLERY

SEQ ID NO: 10 - protein, 118 aa, synthetic construct
EVQLVESGGGLVQPGGSLRLSCAASGFTFSDSWIHWVRQAPGKGLEWVGWISPYGGSTYYADSYRSRFTISADTSKNTAYLQMNSLRAEDTAVYYCARRHWPGGFDYWGQGTLVTVSS

SEQ ID NO: 11 - protein, 116 aa, synthetic construct
QVQLQESGPGLVKPSETLSLTCTVSGGSLDNYYWSWIRQPPGKGLEWIGYIYYSGNTNYNPSLKSRVTISVDTSKNQFSLKLSSVTAADTAVYYCARGGRFLERYWGQGTLVTVSS

SEQ ID NO: 12 - protein, 107 aa, synthetic construct
EIVLTQSPSSLSASVGDRVTITCLASQTIGTWLAWYQQKPGKSPQLLIYAASTLQSGVPSRFSGSGSGTDFTLTISSLQPEDVATYYCQQYYSTPRTFGQGTKVEIK

SEQ ID NO: 13 - protein, 330 aa, synthetic construct
ASTKGPSVFPLAPSSKSTSGGTAALGCLVKDYFPEPVTVSWNSGALTSGVHTFPAVLQSSGLYSLSSVVTVPSSSLGTQTYICNVNHKPSNTKVDKKVEPKSCDKTHTCPPCPAPELLGGPSVFLFPPKPKDTLMISRTPEVTCVVVDVSHEDPEVKFNWYVDGVEVHNAKTKPREEQYASTYRVVSVLTVLHQDWLNGKEYKCKVSNKALPAPIEKTISKAKGQPREPQVYTLPPCRDELTKNQVSLWCLVKGFYPSDIAVEWESNGQPENNYKTTPPVLDSDGSFFLYSKLTVDKSRWQQGNVFSCSVMHEALHNHYTQKSLSLSPGK

SEQ ID NO: 14 - protein, 107 aa, synthetic construct [sequence omitted]

SEQ ID NO: 15 - protein, 330 aa, synthetic construct
ASTKGPSVFPLAPSSKSTSGGTAALGCLVKDYFPEPVTVSWNSGALTSGVHTFPAVLQSSGLYSLSSVVTVPSSSLGTQTYICNVNHKPSNTKVDKKVEPKSCDKTHTCPPCPAPELLGGPSVFLFPPKPKDTLMISRTPEVTCVVVDVSHEDPEVKFNWYVDGVEVHNAKTKPREEQYASTYRVVSVLTVLHQDWLNGKEYKCKVSNKALPAPIEKTISKAKGQPREPQVCTLPPSRDELTKNQVSLSCAVKGFYPSDIAVEWESNGQPENNYKTTPPVLDSDGSFFLVSKLTVDKSRWQQGNVFSCSVMHEALHNHYTQKSLSLSPGK

SEQ ID NO: 16 - protein, 448 aa, synthetic construct
EVQLVESGGGLVQPGGSLRLSCAASGFTFSDSWIHWVRQAPGKGLEWVGWISPYGGSTYYADSYRSRFTISADTSKNTAYLQMNSLRAEDTAVYYCARRHWPGGFDYWGQGTLVTVSSASTKGPSVFPLAPSSKSTSGGTAALGCLVKDYFPEPVTVSWNSGALTSGVHTFPAVLQSSGLYSLSSVVTVPSSSLGTQTYICNVNHKPSNTKVDKKVEPKSCDKTHTCPPCPAPELLGGPSVFLFPPKPKDTLMISRTPEVTCVVVDVSHEDPEVKFNWYVDGVEVHNAKTKPREEQYASTYRVVSVLTVLHQDWLNGKEYKCKVSNKALPAPIEKTISKAKGQPREPQVYTLPPCRDELTKNQVSLWCLVKGFYPSDIAVEWESNGQPENNYKTTPPVLDSDGSFFLYSKLTVDKSRWQQGNVFSCSVMHEALHNHYTQKSLSLSPGK

SEQ ID NO: 17 - protein, 446 aa, synthetic construct
QVQLQESGPGLVKPSETLSLTCTVSGGSLDNYYWSWIRQPPGKGLEWIGYIYYSGNTNYNPSLKSRVTISVDTSKNQFSLKLSSVTAADTAVYYCARGGRFLERYWGQGTLVTVSSASTKGPSVFPLAPSSKSTSGGTAALGCLVKDYFPEPVTVSWNSGALTSGVHTFPAVLQSSGLYSLSSVVTVPSSSLGTQTYICNVNHKPSNTKVDKKVEPKSCDKTHTCPPCPAPELLGGPSVFLFPPKPKDTLMISRTPEVTCVVVDVSHEDPEVKFNWYVDGVEVHNAKTKPREEQYASTYRVVSVLTVLHQDWLNGKEYKCKVSNKALPAPIEKTISKAKGQPREPQVCTLPPSRDELTKNQVSLSCAVKGFYPSDIAVEWESNGQPENNYKTTPPVLDSDGSFFLVSKLTVDKSRWQQGNVFSCSVMHEALHNHYTQKSLSLSPGK

SEQ ID NO: 18 - protein, 214 aa, synthetic construct
EIVLTQSPSSLSASVGDRVTITCLASQTIGTWLAWYQQKPGKSPQLLIYAASTLQSGVPSRFSGSGSGTDFTLTISSLQPEDVATYYCQQYYSTPRTFGQGTKVEIKRTVAAPSVFIFPPSDEQLKSGTASVVCLLNNFYPREAKVQWKVDNALQSGNSQESVTEQDSKDSTYSLSSTLTLSKADYEKHKVYACEVTHQGLSSPVTKSFNRGEC

SEQ ID NO: 19 - protein, 330 aa, synthetic construct
ASTKGPSVFPLAPSSKSTSGGTAALGCLVKDYFPEPVTVSWNSGALTSGVHTFPAVLQSSGLYSLSSVVTVPSSSLGTQTYICNVNHKPSNTKVDKKVEPKSCDKTHTCPPCPAPELLGGPSVFLFPPKPKDTLMISRTPEVTCVVVDVSHEDPEVKFNWYVDGVEVHNAKTKPREEQYNSTYRVVSVLTVLHQDWLNGKEYKCKVSNKALPAPIEKTISKAKGQPREPQVYTLPPCRDELTKNQVSLWCLVKGFYPSDIAVEWESNGQPENNYKTTPPVLDSDGSFFLYSKLTVDKSRWQQGNVFSCSVMHEALHNHYTQKSLSLSPGK

SEQ ID NO: 20 - protein, 330 aa, synthetic construct
ASTKGPSVFPLAPSSKSTSGGTAALGCLVKDYFPEPVTVSWNSGALTSGVHTFPAVLQSSGLYSLSSVVTVPSSSLGTQTYICNVNHKPSNTKVDKKVEPKSCDKTHTCPPCPAPELLGGPSVFLFPPKPKDTLMISRTPEVTCVVVDVSHEDPEVKFNWYVDGVEVHNAKTKPREEQYNSTYRVVSVLTVLHQDWLNGKEYKCKVSNKALPAPIEKTISKAKGQPREPQVCTLPPSRDELTKNQVSLSCAVKGFYPSDIAVEWESNGQPENNYKTTPPVLDSDGSFFLVSKLTVDKSRWQQGNVFSCSVMHEALHNHYTQKSLSLSPGK

SEQ ID NO: 21 - protein, 448 aa, synthetic construct
EVQLVESGGGLVQPGGSLRLSCAASGFTFSDSWIHWVRQAPGKGLEWVGWISPYGGSTYYADSYRSRFTISADTSKNTAYLQMNSLRAEDTAVYYCARRHWPGGFDYWGQGTLVTVSSASTKGPSVFPLAPSSKSTSGGTAALGCLVKDYFPEPVTVSWNSGALTSGVHTFPAVLQSSGLYSLSSVVTVPSSSLGTQTYICNVNHKPSNTKVDKKVEPKSCDKTHTCPPCPAPELLGGPSVFLFPPKPKDTLMISRTPEVTCVVVDVSHEDPEVKFNWYVDGVEVHNAKTKPREEQYNSTYRVVSVLTVLHQDWLNGKEYKCKVSNKALPAPIEKTISKAKGQPREPQVYTLPPCRDELTKNQVSLWCLVKGFYPSDIAVEWESNGQPENNYKTTPPVLDSDGSFFLYSKLTVDKSRWQQGNVFSCSVMHEALHNHYTQKSLSLSPGK

SEQ ID NO: 22 - protein, 446 aa, synthetic construct
QVQLQESGPGLVKPSETLSLTCTVSGGSLDNYYWSWIRQPPGKGLEWIGYIYYSGNTNYNPSLKSRVTISVDTSKNQFSLKLSSVTAADTAVYYCARGGRFLERYWGQGTLVTVSSASTKGPSVFPLAPSSKSTSGGTAALGCLVKDYFPEPVTVSWNSGALTSGVHTFPAVLQSSGLYSLSSVVTVPSSSLGTQTYICNVNHKPSNTKVDKKVEPKSCDKTHTCPPCPAPELLGGPSVFLFPPKPKDTLMISRTPEVTCVVVDVSHEDPEVKFNWYVDGVEVHNAKTKPREEQYNSTYRVVSVLTVLHQDWLNGKEYKCKVSNKALPAPIEKTISKAKGQPREPQVCTLPPSRDELTKNQVSLSCAVKGFYPSDIAVEWESNGQPENNYKTTPPVLDSDGSFFLVSKLTVDKSRWQQGNVFSCSVMHEALHNHYTQKSLSLSPGK